European Patent Application EP 4 455 164 A1, published October 30, 2024. Title: ANTI-FRα ANTIBODY, AND ANTIBODY-DRUG CONJUGATE AND USE THEREOF. Applicant: Bio-Thera Solutions, Ltd. Application CN PCT/CN2022/141572, filed December 23, 2022. The sequence listing filed with the application follows.

SEQUENCE LISTING (35 sequences)

SEQ ID NO: 1 - protein, 30 aa, synthetic construct
QVQLVQSGVEVKKPGASVKVSCKASGYTFT

SEQ ID NO: 2 - protein, 14 aa, synthetic construct
WVRQAPGQGLEWMG

SEQ ID NO: 3 - protein, 32 aa, synthetic construct
RVTLTTDSSTTTAYMELKSLQFDDTAVYYCAR

SEQ ID NO: 4 - protein, 32 aa, synthetic construct
GVPARFSGSGSGTDFTLTISSLEPEDFAVYYC

SEQ ID NO: 5 - protein, 5 aa, synthetic construct
GYFMN

SEQ ID NO: 6 - protein, 17 aa, synthetic construct
RIHPYDGDTFYNQNFKD

SEQ ID NO: 7 - protein, 9 aa, synthetic construct
YDGSRAMDY

SEQ ID NO: 8 - protein, 15 aa, synthetic construct
KASQSVSFAGTSLMH

SEQ ID NO: 9 - protein, 7 aa, synthetic construct
RASNLEA

SEQ ID NO: 10 - protein, 9 aa, synthetic construct
QQSREYPYT

SEQ ID NO: 11 - protein, 11 aa, synthetic construct
WGQGTTVTVSS

SEQ ID NO: 12 - protein, 23 aa, synthetic construct
EIVLTQSPATLSLSPGERATLSC

SEQ ID NO: 13 - protein, 15 aa, synthetic construct
WYQQKPGQAPRLLIY

SEQ ID NO: 14 - protein, 10 aa, synthetic construct
FGGGTKVEIK

SEQ ID NO: 15 - protein, 118 aa, synthetic construct
QVQLVQSGVEVKKPGASVKVSCKASGYSFTGYFMNWVRQAPGQGLEWIGRIHPYDGDTFYNQNFKDKATLTVDKSTTTAYMELKSLQFDDTAVYYCTRYDGSRAMDYWGQGTTVTVSS

SEQ ID NO: 16 - protein, 111 aa, synthetic construct
EIVLTQSPATLSLSPGERATLSCKASQSVSFAGTSLMHWYQQKPGQAPRLLIYRASNLEAGVPARFSGSGSKTDFTLTISSLEPEDFAVYYCQQSREYPYTFGGGTKVEIK

SEQ ID NO: 17 - protein, 330 aa, synthetic construct [sequence omitted]

SEQ ID NO: 18 - protein, 107 aa, synthetic construct [sequence omitted]

SEQ ID NO: 19 - protein, 448 aa, synthetic construct
QVQLVQSGVEVKKPGASVKVSCKASGYSFTGYFMNWVRQAPGQGLEWIGRIHPYDGDTFYNQNFKDKATLTVDKSTTTAYMELKSLQFDDTAVYYCTRYDGSRAMDYWGQGTTVTVSSASTKGPSVFPLAPSSKSTSGGTAALGCLVKDYFPEPVTVSWNSGALTSGVHTFPAVLQSSGLYSLSSVVTVPSSSLGTQTYICNVNHKPSNTKVDKKVEPKSCDKTHTCPPCPAPELLGGPSVFLFPPKPKDTLMISRTPEVTCVVVDVSHEDPEVKFNWYVDGVEVHNAKTKPREEQYNSTYRVVSVLTVLHQDWLNGKEYKCKVSNKALPAPIEKTISKAKGQPREPQVYTLPPSRDELTKNQVSLTCLVKGFYPSDIAVEWESNGQPENNYKTTPPVLDSDGSFFLYSKLTVDKSRWQQGNVFSCSVMHEALHNHYTQKSLSLSPGK

SEQ ID NO: 20 - protein, 218 aa, synthetic construct
EIVLTQSPATLSLSPGERATLSCKASQSVSFAGTSLMHWYQQKPGQAPRLLIYRASNLEAGVPARFSGSGSKTDFTLTISSLEPEDFAVYYCQQSREYPYTFGGGTKVEIKRTVAAPSVFIFPPSDEQLKSGTASVVCLLNNFYPREAKVQWKVDNALQSGNSQESVTEQDSKDSTYSLSSTLTLSKADYEKHKVYACEVTHQGLSSPVTKSFNRGEC

SEQ ID NO: 21 - protein, 19 aa, synthetic construct
MDWTWRILFLVAAATGAHS

SEQ ID NO: 22 - protein, 20 aa, synthetic construct
MEAPAQLLFLLLLWLPDTTG

SEQ ID NO: 23 - DNA, 1347 bp, synthetic construct
  source 1..1347: mol_type = other DNA
caggtgcagctggtgcagtccggcgtggaggtgaagaagcccggcgccagcgtgaaggtgagctgcaaggcctccggctactccttcaccggctacttcatgaactgggtgaggcaggcccccggccagggactggaatggatcggcagaatccacccctacgacggcgacaccttttacaatcagaacttcaaggataaggccaccctgaccgtggataagtccaccaccaccgcctacatggagctgaagtccctgcagtttgacgataccgccgtgtactactgtaccagatacgacggctccagagccatggactactggggccagggcaccaccgtgaccgtgtcctccgccagcaccaagggcccatcggtcttccccctggcaccctcctccaagagcacctctgggggcacagcggccctgggctgcctggtcaaggactacttccccgaaccggtgacggtgtcgtggaactcaggcgccctgaccagcggcgtgcacaccttcccggctgtcctacagtcctcaggactctactccctcagcagcgtggtgaccgtgccctccagcagcttgggcacccagacctacatctgcaacgtgaatcacaagcccagcaacaccaaggtggacaagaaagttgagcccaaatcttgtgacaaaactcacacatgcccaccgtgcccagcacctgaactcctggggggaccgtcagtcttcctcttccccccaaaacccaaggacaccctcatgatctcccggacccctgaggtcacatgcgtggtggtggacgtgagccacgaagaccctgaggtcaagttcaactggtacgtggacggcgtggaggtgcataatgccaagacaaagccgcgggaggagcagtacaacagcacgtaccgtgtggtcagcgtcctcaccgtcctgcaccaggactggctgaatggcaaggagtacaagtgcaaggtctccaacaaagccctcccagcccccatcgagaaaaccatctccaaagccaaagggcagccccgagaaccacaggtgtacaccctgcccccatcccgggatgagctgaccaagaaccaggtcagcctgacctgcctggtcaaaggcttctatcccagcgacatcgccgtggagtgggagagcaatgggcagccggagaacaactacaagaccacgcctcccgtgctggactccgacggctccttcttcctctacagcaagctcaccgtggacaagagcaggtggcagcaggggaacgtcttctcatgctccgtgatgcatgaggctctgcacaaccactacacgcagaagagcctctccctgtctccgggtaaatga

SEQ ID NO: 24 - DNA, 657 bp, synthetic construct
  source 1..657: mol_type = other DNA
gagatcgtgctgacccagtcccccgccaccctgagcctgagcccaggagagagggccaccctgtcctgcaaggcctcccagagcgtgagctttgccggcaccagcctgatgcactggtatcaacagaagcccggccaggcccctaggctgctgatctacagagccagcaacctggaggccggcgtgcctgctaggttttccggcagcggctccaagaccgatttcaccctgaccatcagcagcctggagcctgaggattttgccgtgtactactgccagcagtccagggagtacccctacaccttcggcggcggcaccaaggtggagatcaagcgtacggtggctgcaccatctgtcttcatcttcccgccatctgatgagcagttgaaatctggaactgcctctgttgtgtgcctgctgaataacttctatcccagagaggccaaagtacagtggaaggtggataacgccctccaatcgggtaactcccaggagagtgtcacagagcaggacagcaaggacagcacctacagcctcagcagcaccctgacgctgagcaaagcagactacgagaaacacaaagtctacgcctgcgaagtcacccatcagggcctgagctcgcccgtcacaaagagcttcaacaggggagagtgttga

SEQ ID NO: 25 - DNA, 57 bp, synthetic construct
  source 1..57: mol_type = other DNA
atggattggacctggagaatcctgttcctggtggccgccgccaccggcgctcattct

SEQ ID NO: 26 - DNA, 60 bp, synthetic construct
  source 1..60: mol_type = other DNA
atggaggcccctgcccagctgctgttcctgctgctgctgtggctgcctgataccaccggc

SEQ ID NO: 27 - protein, 233 aa, synthetic construct
MAQRMTTQLLLLLVWVAVVGEAQTRIAWARTELLNVCMNAKHHKEKPGPEDKLHEQCRPWRKNACCSTNTSQEAHKDVSYLYRFNWNHCGEMAPACKRHFIQDTCLYECSPNLGPWIQQVDQSWRKERVLNVPLCKEDCEQWWEDCRTSYTCKSNWHKGWNWTSGFNKCAVGAACQPFHFYFPTPTVLCNEIWTHSYKVSNYSRGSGRCIQMWFDPAQGNPNEEVARFYAAAM

SEQ ID NO: 28 - protein, 241 aa, synthetic construct
MAQRMTTQLLLLLVWVAVVGEAQTRIAWARTELLNVCMNAKHHKEKPGPEDKLHEQCRPWRKNACCSTNTSQEAHKDVSYLYRFNWNHCGEMAPACKRHFIQDTCLYECSPNLGPWIQQVDQSWRKERVLNVPLCKEDCEQWWEDCRTSYTCKSNWHKGWNWTSGFNKCAVGAACQPFHFYFPTPTVLCNEIWTHSYKVSNYSRGSGRCIQMWFDPAQGNPNEEVARFYAAAMHHHHHHHH

SEQ ID NO: 29 - protein, 30 aa, synthetic construct
QVQLVQSGVEVKKPGASVKVSCKASGYSFT

SEQ ID NO: 30 - protein, 14 aa, synthetic construct
WVRQAPGQGLEWIG

SEQ ID NO: 31 - protein, 32 aa, synthetic construct
KATLTVDKSTTTAYMELKSLQFDDTAVYYCTR

SEQ ID NO: 32 - protein, 32 aa, synthetic construct
GVPARFSGSGSKTDFTLTISSLEPEDFAVYYC

SEQ ID NO: 33 - skipped

SEQ ID NO: 34 - protein, 448 aa, synthetic construct
QVQLVQSGAEVVKPGASVKISCKASGYTFTGYFMNWVKQSPGQSLEWIGRIHPYDGDTFYNQKFQGKATLTVDKSSNTAHMELLSLTSEDFAVYYCTRYDGSRAMDYWGQGTTVTVSSASTKGPSVFPLAPSSKSTSGGTAALGCLVKDYFPEPVTVSWNSGALTSGVHTFPAVLQSSGLYSLSSVVTVPSSSLGTQTYICNVNHKPSNTKVDKKVEPKSCDKTHTCPPCPAPELLGGPSVFLFPPKPKDTLMISRTPEVTCVVVDVSHEDPEVKFNWYVDGVEVHNAKTKPREEQYNSTYRVVSVLTVLHQDWLNGKEYKCKVSNKALPAPIEKTISKAKGQPREPQVYTLPPSRDELTKNQVSLTCLVKGFYPSDIAVEWESNGQPENNYKTTPPVLDSDGSFFLYSKLTVDKSRWQQGNVFSCSVMHEALHNHYTQKSLSLSPGK

SEQ ID NO: 35 - protein, 218 aa, synthetic construct
DIVLTQSPLSLAVSLGQPAIISCKASQSVSFAGTSLMHWYHQKPGQQPRLLIYRASNLEAGVPDRFSGSGSKTDFTLTISPVEAEDAATYYCQQSREYPYTFGGGTKLEIKRTVAAPSVFIFPPSDEQLKSGTASVVCLLNNFYPREAKVQWKVDNALQSGNSQESVTEQDSKDSTYSLSSTLTLSKADYEKHKVYACEVTHQGLSSPVTKSFNRGEC